European Patent Specification EP 4 050 023 B1, published March 13, 2024. Title: Novel ABC transporter ATP-binding protein variant and a method for producing L-lysine using the same. Applicant: CJ CheilJedang Corporation. The sequence listing filed with the application follows.

SEQUENCE LISTING (11 sequences)

SEQ ID NO: 1 - protein, 269 aa, Artificial Sequence
  (V199M)_ABC transporter ATP-binding protein
MTTNHQLSAEEISLAYGERTIIDSLSVDIVPGKITSIVGPNGCGKSTLLRAFARLLKPSAGQALIDAHPLPSLPGKELARMLGLLPQSPTAPEGIVVADLVGRGRHPHQGLMGRWSTRDYEVVAQALEMTNTTELAERPIDELSGGQRQRVWIAMALAQETDILLLDEPTTYLDIANQLEVLDLLTDLNHNHGTTIVMMLHELGLAARYSDHLIAMNAGKIYAQGTPTNVITETMMSEVFHTDARIIADPVSGAPLVMPMGRHHITALH

SEQ ID NO: 2 - DNA, 810 bp, Artificial Sequence
  (V199M)_NCgl0636
gtgaccaccaaccatcaactatccgccgaagaaatttccctggcgtacggcgagcgcaccatcatcgattcgctcagcgtcgacatcgtccccggcaaaatcacctccatcgtcggccccaacggatgcggcaaatcaacgctgctgcgcgcctttgcgcgcctccttaaacctagcgccgggcaagcgcttatcgacgcccacccccttccttcactgccaggcaaagaactagctcgcatgctcgggctgttaccgcaatcccccaccgcacctgaaggcatcgtcgtcgccgacctcgtgggccgcggccgccacccccaccaaggactcatgggcagatggtccacacgcgactacgaagtagtggcccaagcattggaaatgaccaacaccaccgagcttgccgaacgccccatcgacgaactctccggcggccaacgccaacgcgtctggatcgccatggcccttgcccaagaaacagacatcctgcttcttgatgaacccaccacctacctcgacatcgccaaccagctcgaagtgcttgatctcctcactgacctcaaccacaaccacggcaccaccatcgtcatgatgctccacgaattgggacttgccgcacgttactctgaccacctcatcgccatgaacgccggaaaaatctacgcccaaggcacccccaccaacgtcatcaccgaaaccatgatgagcgaggtcttccacaccgacgcccgcattatcgccgacccagtctccggcgcaccactggtcatgcccatgggacgacaccacatcaccgcacttcactag

SEQ ID NO: 3 - protein, 269 aa, Artificial Sequence
  (WT)_ABC transporter ATP-binding protein
MTTNHQLSAEEISLAYGERTIIDSLSVDIVPGKITSIVGPNGCGKSTLLRAFARLLKPSAGQALIDAHPLPSLPGKELARMLGLLPQSPTAPEGIVVADLVGRGRHPHQGLMGRWSTRDYEVVAQALEMTNTTELAERPIDELSGGQRQRVWIAMALAQETDILLLDEPTTYLDIANQLEVLDLLTDLNHNHGTTIVMVLHELGLAARYSDHLIAMNAGKIYAQGTPTNVITETMMSEVFHTDARIIADPVSGAPLVMPMGRHHITALH

SEQ ID NO: 4 - DNA, 810 bp, Artificial Sequence
  (WT)_NCgl0636
gtgaccaccaaccatcaactatccgccgaagaaatttccctggcgtacggcgagcgcaccatcatcgattcgctcagcgtcgacatcgtccccggcaaaatcacctccatcgtcggccccaacggatgcggcaaatcaacgctgctgcgcgcctttgcgcgcctccttaaacctagcgccgggcaagcgcttatcgacgcccacccccttccttcactgccaggcaaagaactagctcgcatgctcgggctgttaccgcaatcccccaccgcacctgaaggcatcgtcgtcgccgacctcgtgggccgcggccgccacccccaccaaggactcatgggcagatggtccacacgcgactacgaagtagtggcccaagcattggaaatgaccaacaccaccgagcttgccgaacgccccatcgacgaactctccggcggccaacgccaacgcgtctggatcgccatggcccttgcccaagaaacagacatcctgcttcttgatgaacccaccacctacctcgacatcgccaaccagctcgaagtgcttgatctcctcactgacctcaaccacaaccacggcaccaccatcgtcatggtgctccacgaattgggacttgccgcacgttactctgaccacctcatcgccatgaacgccggaaaaatctacgcccaaggcacccccaccaacgtcatcaccgaaaccatgatgagcgaggtcttccacaccgacgcccgcattatcgccgacccagtctccggcgcaccactggtcatgcccatgggacgacaccacatcaccgcacttcactag

SEQ ID NO: 5 - DNA, 36 bp, Artificial Sequence
  NCgl0636_1F
tcgagctcggtacccggccccaacggatgcggcaaa

SEQ ID NO: 6 - DNA, 44 bp, Artificial Sequence
  NCgl0636_2R
aagtcccaattcgtggagcatcatgacgatggtggtgccgtggt

SEQ ID NO: 7 - DNA, 44 bp, Artificial Sequence
  NCgl0636_3F
accacggcaccaccatcgtcatgatgctccacgaattgggactt

SEQ ID NO: 8 - DNA, 36 bp, Artificial Sequence
  NCgl0636_4R
ctctagaggatccccagtaggtgcgcatgacgccgc

SEQ ID NO: 9 - DNA, 21 bp, Artificial Sequence
  NCgl0636_5F
ggccccaacggatgcggcaaa

SEQ ID NO: 10 - DNA, 21 bp, Artificial Sequence
  NCgl0636_6R
agtaggtgcgcatgacgccgc

SEQ ID NO: 11 - DNA, 5803 bp, Artificial Sequence
  pDCM2_plasmid
gttcgcttgctgtccataaaaccgcccagtctagctatcgccatgtaagcccactgcaagctacctgctttctctttgcgcttgcgttttcccttgtccagatagcccagtagctgacattcatccggggtcagcaccgtttctgcggactggctttctacgtgttccgcttcctttagcagcccttgcgccctgagtgcttgcggcagcgtgaagctagcttttatcgccattcgccattcaggctgcgcaactgttgggaagggcgatcggtgcgggcctcttcgctattacgccagctggcgaaagggggatgtgctgcaaggcgattaagttgggtaacgccagggttttcccagtcacgacgttgtaaaacgacggccagtgaattcgagctcggtacccggggatcctctagagtcgacctgcaggcatgcaagcttggcgtaatcatggtcatagctgtttcctgtgtgaaattgttatccgctcacaattccacacaacatacgagccggaagcataaagtgtaaagcctggggtgcctaatgagtgagctaactcacattaattgcgttgcgctcactgcccgctttccagtcgggaaacctgtcgtgccagctgcattaatgaatcggccaacgcgcggggagaggcggtttgcgtattgggcgctcttccgcttcctcgctcactgactcgctgcgctcggtcgttcggctgcggcgagcggtatcagctcactcaaaggcggtaatacggttatccacagaatcaggggataacgcaggaaagaacatgtgagcaaaaggccagcaaaaggccaggaaccgtaaaaaggccgcgttgctggcgtttttccataggctccgcccccctgacgagcatcacaaaaatcgacgctcaagtcagaggtggcgaaacccgacaggactataaagataccaggcgtttccccctggaagctccctcgtgcgctctcctgttccgaccctgccgcttaccggatacctgtccgcctttctcccttcgggaagcgtggcgctttctcaatgctcacgctgtaggtatctcagttcggtgtaggtcgttcgctccaagctgggctgtgtgcacgaaccccccgttcagcccgaccgctgcgccttatccggtaactatcgtcttgagtccaacccggtaagacacgacttatcgccactggcagcagccactggtaacaggattagcagagcgaggtatgtaggcggtgctacagagttcttgaagtggtggcctaactacggctacactagaaggacagtatttggtatctgcgctctgctgaagccagttaccttcggaaaaagagttggtagctcttgatccggcaaacaaaccaccgctggtagcggtggtttttttgtttgcaagcagcagattacgcgcagaaaaaaaggatctcaagaagatcctttgatcttttctacggggtctgacgctcagtggaacgaaaactcacgttaagggattttggtcatgagattatcaaaaaggatcttcacctagatccttttggggtgggcgaagaactccagcatgagatccccgcgctggaggatcatccagccctgatagaaacagaagccactggagcacctcaaaaacaccatcatacactaaatcagtaagttggcagcatcacccgacgcactttgcgccgaataaatacctgtgacggaagatcacttcgcagaataaataaatcctggtgtccctgttgataccgggaagccctgggccaacttttggcgaaaatgagacgttgatcggcacgtaagaggttccaactttcaccataatgaaataagatcactaccgggcgtattttttgagttatcgagattttcaggagctgatagaaacagaagccactggagcacctcaaaaacaccatcatacactaaatcagtaagttggcagcatcacccgacgcactttgcgccgaataaatacctgtgacggaagatcacttcgcagaataaataaatcctggtgtccctgttgataccgggaagccctgggccaacttttggcgaaaatgagacgttgatcggcacgtaagaggttccaactttcaccataatgaaataagatcactaccgggcgtattttttgagttatcgagattttcaggagctctttggcatcgtctctcgcctgtcccctcagttcagtaatttcctgcatttgcctgtttccagtcggtagatattccacaaaacagcagggaagcagcgcttttccgctgcataaccctgcttcggggtcattatagcgattttttcggtatatccatcctttttcgcacgatatacaggattttgccaaagggttcgtgtagactttccttggtgtatccaacggcgtcagccgggcaggataggtgaagtaggcccacccgcgagcgggtgttccttcttcactgtcccttattcgcacctggcggtgctcaacgggaatcctgctctgcgaggctggccggctaccgccggcgtaacagatgagggcaagcggatggctgatgaaaccaagccaaccaggaagggcagcccacctatcaaggtgtactgccttccagacgaacgaagagcgattgaggaaaaggcggcggcggccggcatgagcctgtcggcctacctgctggccgtcggccagggctacaaaatcacgggcgtcgtggactatgagcacgtccgcgagggcgtcccggaaaacgattccgaagcccaacctttcatagaaggcggcggtggaatcgaaatctcgtgatggcaggttgggcgtcgcttggtcggtcatttcgaaaaaggttaggaatacggttagccatttgcctgcttttatatagttcantatgggattcacctttatgttgataagaaataaaagaaaatgccaataggatatcggcattttcttttgcgtttttatttgttaactgttaattgtccttgttcaaggatgctgtctttgacaacagatgttttcttgcctttgatgttcagcaggaagctcggcgcaaacgttgattgtttgtctgcgtagaatcctctgtttgtcatatagcttgtaatcacgacattgtttcctttcgcttgaggtacagcgaagtgtgagtaagtaaaggttacatcgttaggcggatcaagatccatttttaacacaaggccagttttgttcagcggcttgtatgggccagttaaagaattagaaacataaccaagcatgtaaatatcgttagacgtaatgccgtcaatcgtcatttttgatccgcgggagtcagtgaacaggtaccatttgccgttcattttaaagacgttcgcgcgttcaatttcatctgttactgtgttagatgcaatcagcggtttcatcacttttttcagtgtgtaatcatcgtttagctcaatcataccgagagcgccgtttgctaactcagccgtgcgttttttatcgctttgcagaagtttttgactttcttgacggaagaatgatgtgcttttgccatagtatgctttgttaaataaagattcttcgccttggtagccatcttcagttccagtgtttgcttcaaatactaagtatttgtggcctttatcttctacgtagtgaggatctctcagcgtatggttgtcgcctgagctgtagttgccttcatcgatgaactgctgtacattttgatacgtttttccgtcaccgtcaaagattgatttataatcctctacaccgttgatgttcaaagagctgtctgatgctgatacgttaacttgtgcagttgtcagtgtttgtttgccgtaatgtttaccggagaaatcagtgtagaataaacggatttttccgtcagatgtaaatgtggctgaacctgaccattcttgtgtttggtcttttaggatagaatcatttgcatcgaatttgtcgctgtctttaaagacgcggccagcgtttttccagctgtcaatagaagtttcgccgactttttgatagaacatgtaaatcgatgtgtcatccgcatttttaggatctccggctaatgcaaagacgatgtggtagccgtgatagtttgcgacagtgccgtcagcgttttgtaatggccagctgtcccaaacgtccaggccttttgcagaagagatatttttaattgtggacgaatcaaattcagaaacttgatatttttcatttttttgctgttcagggatttgcagcatatcatggcgtgtaatatgggaaatgccgtatgtttccttatatggcttttggttcgtttctttcgcaaacgcttgagttgcgcctcctgccagcagtgcggtagtaaaggttaatactgttgcttgttttgcaaactttttgatgttcatcgttcatgtctccttttttatgtactgtgttagcggtctgcttcttccagccctcctgtttgaagatggcaagttagttacgcacaataaaaaaagacctaaaatatgtaaggggtgacgccaaagtatacactttgccctttacacattttaggtcttgcctgctttatcagtaacaaacccgcgcgatttacttttcgacctcattctattagactctcgtttggattgcaactggtctattttcctcttttgtttgatagaaaatcataaaaggatttgcagactacgggcctaaagaactaaaaaatctatctgtttcttttcattctctgtattttttatagtttctgttgcatgggcataaagttgcctttttaatcacaattcagaaaatatcataatatctcatttcactaaataatagtgaacggcaggtatatgtgatgggttaaaaaggatcaccccagagtcccgctcagaagaactcgtcaagaaggcgatagaaggcgatgcgctgcgaatcgggagcggcgataccgtaaagcacgaggaagcggtcagcccattcgccgccaagctcttcagcaatatcacgggtagccaacgctatgtcctgatagcggtccgccacacccagccggccacagtcgatgaatccagaaaagcggccattttccaccatgatattcggcaagcaggcatcgccatgggtcacgacgagatcctcgccgtcgggcatccgcgccttgagcctggcgaacagttcggctggcgcgagcccctgatgctcttcgtccagatcatcctgatcgacaagaccggcttccatccgagtacgtgctcgctcgatgcgatgtttcgcttggtggtcgaatgggcaggtagccggatcaagcgtatgcagccgccgcattgcatcagccatgatggatactttctcggcaggagcaaggtgagatgacaggagatcctgccccggcacttcgcccaatagcagccagtcccttcccgcttcagtgacaacgtcgagacagctgcgcaaggaacgcccgtcgtggccagccacgatagccgcgctgcctcgtcttggagttcattcagggcaccggacaggtcggtcttgacaaaaagaaccgggcgcccctgcgctgacagccggaacacggcggcatcagagcagccgattgtctgttgtgcccagtcatagccgaatagcctctccacccaagcggccggagaacctgcgtgcaatccatcttgttcaatcatgcgaaacgatcctcatcctgtctcttgatcagatcttgatcccctgcgccatcagatccttggcggcaagaaagccatccagtttactttgcagggcttcccaaccttaccagagggcgccccagctggcaattccg